European Patent Application EP 4 717 766 A1, published April 1, 2026. Title: 树突状细胞靶向的类病毒体DVLP及其制备方法和应用. Applicant: 上海本导基因技术有限公司. Application CN. The sequence listing filed with the application follows.

SEQUENCE LISTING (18 sequences)

SEQ ID NO: 1 - protein, 985 aa, synthetic construct
MSAAPLVTAMCLLGNVSFPCDRPPTCYTREPSRALDILEENVNHEAYDTLLNAILRCGSSGSVIDDFTLTSPYLGTCSYCHHTVPCFSPVKIEQVWDEADDNTIRIQTSAQFGYDQSGAASANKYRYMAAAAYPYDVPDYATVKEGTMDDIKISTSGPCRRLSYKGYFLLAKCPPGDSVTVSIVSSNSATSCTLARKIKPKFVGREKYDLPPVHGKKIPCTVYDRLAATTAGYITMHRPRPHAYTSYLEESSGKVYAKPPSGKNITYECKCGDYKTGTVSTRTEITGCTAIKQCVAYKSDQTKWVFNSPDLIRHDDHTAQGKLHLPFKLIPSTCMVPVAHAPNVIHGFKHISLQLDTDHLTLLTTRRLGANPEPTTEWIVGKTVRNFTVDRDGLEYIWGNHEPVRVYAQESAPGDPHGWPHEIVQHYYHRHPVYTILAVASATVAMMIGVTVAVLCACKARRECLTPYALAPNAVIPTSLALLCCVRSANAETFTETMSYLWSNSQPFFWVQLCIPLAAFIVLMRCCSCCLPFLVVAGAYLAKVDAYEHATTVPNVPQIPYKALVERAGYAPLNLEITVMSSEVLPSTNQEYITCKFTTVVPSPKIKCCGSLECQPAAHADYTCKVFGGVYPFMWGGAQCFCDSENSQMSEAYVELSADCASDHAQAIKVHTAAMKVGLRIVYGNTTSFLDVYVNGVTPGTSKDLKVIAGPISASFTPFDHKVVIHRGLVYNYDFPEYGAMKPGAFGDIQATSLTSKDLIASTDIRLLKPSAKNVHVPYTQASSGFEMWKNNSGRPLQETAPFGCKIAVNPLRAVDCSYGNIPISIDIPNAAFIRTSDAPLVSTVKCEVSECTYSADFGGMATLQYVSDREGQCPVHSHSSTATLQESTVHVLEKGAVTVHFSTASPQANFIVSLCGKKTTCNAECKPPADHIVSTPHKNDQEFQAAISKTSWSWLFALFGGASSLLIIGLMIFACSMMLTSTRR

SEQ ID NO: 2 - DNA, 2958 bp, synthetic construct
  source 1..2958: mol_type = other DNA
atgagcgctgctcctctggtgaccgctatgtgcctgctgggaaacgtgtcttttccttgtgacagaccccccacctgctacaccagagagccttctagagccctggacatcctggaggagaacgtgaaccacgaggcttacgacaccctgctgaacgctatcctgcgctgcggaagcagcggatctgtgatcgacgacttcaccctgacctccccctatctgggcacctgtagctattgccaccacaccgtgccctgctttagccctgtgaagattgagcaggtgtgggacgaggccgacgacaataccattagaatccagaccagcgcccagttcggctatgaccagagcggagctgccagcgctaataaataccggtacatggctgccgccgcctacccttatgatgtgcctgactacgccaccgtgaaggagggaaccatggatgacatcaagatcagcacctccggaccttgtagaagactgagctacaaaggctacttcctgctggccaagtgcccccctggagattctgtgaccgtgagtatcgtgagcagcaacagcgccaccagctgcacactggctagaaaaatcaaaccaaaattcgtgggcagagagaagtacgacctgccacccgtgcacggaaagaagatcccctgcacagtgtacgacagactggccgctaccacagccggatacatcaccatgcacagacccaggccccatgcttacaccagctacctggaagaatcctccggcaaagtgtacgccaaaccccccagcggaaaaaacatcacctacgagtgcaagtgcggcgactacaagaccggcaccgtgagcaccagaaccgagatcaccggctgcaccgccatcaagcagtgcgtggcctacaagagcgaccagaccaagtgggtgttcaacagccccgacctgatcagacacgacgaccacaccgcccagggcaagctgcacctgcccttcaagctgatccccagcacctgcatggtgcccgtggcccacgcccccaacgtgatccacggcttcaagcacatcagcctgcagctggacaccgaccacctgaccctgctgaccaccagaagactgggcgccaaccccgagcccaccaccgagtggatcgtgggcaagaccgtgagaaacttcaccgtggacagagacggcctggagtacatctggggcaaccacgagcccgtgagagtgtacgcccaggagagcgcccccggcgacccccacggctggccccacgagatcgtgcagcactactaccacagacaccccgtgtacaccatcctggccgtggccagcgccaccgtggccatgatgatcggcgtgaccgtggccgtgctgtgcgcctgcaaggccagaagagagtgcctgaccccctacgccctggcccccaacgccgtgatccccaccagcctggccctgctgtgctgcgtgagaagcgccaacgccgagaccttcaccgagaccatgagctacctgtggagcaacagccagcccttcttctgggtgcagctgtgcatccccctggccgccttcatcgtgctgatgagatgctgcagctgctgcctgcccttcctggtggtggccggcgcctacctggccaaggtggacgcctacgagcacgccaccaccgtgcccaacgtgccccagatcccctacaaggccctggtggagagagccggctacgcccccctgaacctggagatcaccgtgatgagcagcgaggtgctgcccagcaccaaccaggagtacatcacctgcaagttcaccaccgtggtgcccagccccaagatcaagtgctgcggcagcctggagtgccagcccgccgcccacgccgactacacctgcaaggtgttcggcggcgtgtaccccttcatgtggggcggcgcccagtgcttctgcgacagcgagaacagccagatgagcgaggcctacgtggagctgagcgccgactgcgccagcgaccacgcccaggccatcaaggtgcacaccgccgccatgaaggtgggcctgagaatcgtgtacggcaacaccaccagcttcctggacgtgtacgtgaacggcgtgacccccggcaccagcaaggacctgaaggtgatcgccggccccatcagcgccagcttcacccccttcgaccacaaggtggtgatccacagaggcctggtgtacaactacgacttccccgagtacggcgccatgaagcccggcgccttcggcgacatccaggccaccagcctgaccagcaaggacctgatcgccagcaccgacatcagactgctgaagcccagcgccaagaacgtgcacgtgccctacacccaggccagcagcggcttcgagatgtggaagaacaacagcggcagacccctgcaggagaccgcccccttcggctgcaagatcgccgtgaaccccctgagagccgtggactgcagctacggcaacatccccatcagcatcgacatccccaacgccgccttcatcagaaccagcgacgcccccctggtgagcaccgtgaagtgcgaggtgagcgagtgcacctacagcgccgacttcggcggcatggccaccctgcagtacgtgagcgacagagagggccagtgccccgtgcacagccacagcagcaccgccaccctgcaggagagcaccgtgcacgtgctggagaagggcgccgtgaccgtgcacttcagcaccgccagcccccaggccaacttcatcgtgagcctgtgcggcaagaagaccacctgcaacgccgagtgcaagccccccgccgaccacatcgtgagcaccccccacaagaacgaccaggagttccaggccgccatcagcaagaccagctggagctggctgttcgccctgttcggcggcgccagcagcctgctgatcatcggcctgatgatcttcgcctgcagcatgatgctgaccagcaccagaagataa

SEQ ID NO: 3 - DNA, 4348 bp, synthetic construct
  source 1..4348: mol_type = other DNA
ggtaccgagctcggatcctgagaacttcagggtgagtctatgggacccttgatgttttctttccccttcttttctatggttaagttcatgtcataggaaggggagaagtaacagggtacacatattgaccaaatcagggtaattttgcatttgtaattttaaaaaatgctttcttcttttaatatacttttttgtttatcttatttctaatactttccctaatctctttctttcagggcaataatgatacaatgtatcatgcctctttgcaccattctaaagaataacagtgataatttctgggttaaggcaatagcaatatttctgcatataaatatttctgcatataaattgtaactgatgtaagaggtttcatattgctaatagcagctacaatccagctaccattctgcttttattttatggttgggataaggctggattattctgagtccaagctaggcccttttgctaatcatgttcatacctcttatcttcctcccacagctcctgggcaacgtgctggtctgtgtgctggcccatcactttggcaaagcacgtgagatctgaattctgacactgccaccatgagcgctgctcctctggtgaccgctatgtgcctgctgggaaacgtgtcttttccttgtgacagaccccccacctgctacaccagagagccttctagagccctggacatcctggaggagaacgtgaaccacgaggcttacgacaccctgctgaacgctatcctgcgctgcggaagcagcggatctgtgatcgacgacttcaccctgacctccccctatctgggcacctgtagctattgccaccacaccgtgccctgctttagccctgtgaagattgagcaggtgtgggacgaggccgacgacaataccattagaatccagaccagcgcccagttcggctatgaccagagcggagctgccagcgctaataaataccggtacatggctgccgccgcctacccttatgatgtgcctgactacgccaccgtgaaggagggaaccatggatgacatcaagatcagcacctccggaccttgtagaagactgagctacaaaggctacttcctgctggccaagtgcccccctggagattctgtgaccgtgagtatcgtgagcagcaacagcgccaccagctgcacactggctagaaaaatcaaaccaaaattcgtgggcagagagaagtacgacctgccacccgtgcacggaaagaagatcccctgcacagtgtacgacagactggccgctaccacagccggatacatcaccatgcacagacccaggccccatgcttacaccagctacctggaagaatcctccggcaaagtgtacgccaaaccccccagcggaaaaaacatcacctacgagtgcaagtgcggcgactacaagaccggcaccgtgagcaccagaaccgagatcaccggctgcaccgccatcaagcagtgcgtggcctacaagagcgaccagaccaagtgggtgttcaacagccccgacctgatcagacacgacgaccacaccgcccagggcaagctgcacctgcccttcaagctgatccccagcacctgcatggtgcccgtggcccacgcccccaacgtgatccacggcttcaagcacatcagcctgcagctggacaccgaccacctgaccctgctgaccaccagaagactgggcgccaaccccgagcccaccaccgagtggatcgtgggcaagaccgtgagaaacttcaccgtggacagagacggcctggagtacatctggggcaaccacgagcccgtgagagtgtacgcccaggagagcgcccccggcgacccccacggctggccccacgagatcgtgcagcactactaccacagacaccccgtgtacaccatcctggccgtggccagcgccaccgtggccatgatgatcggcgtgaccgtggccgtgctgtgcgcctgcaaggccagaagagagtgcctgaccccctacgccctggcccccaacgccgtgatccccaccagcctggccctgctgtgctgcgtgagaagcgccaacgccgagaccttcaccgagaccatgagctacctgtggagcaacagccagcccttcttctgggtgcagctgtgcatccccctggccgccttcatcgtgctgatgagatgctgcagctgctgcctgcccttcctggtggtggccggcgcctacctggccaaggtggacgcctacgagcacgccaccaccgtgcccaacgtgccccagatcccctacaaggccctggtggagagagccggctacgcccccctgaacctggagatcaccgtgatgagcagcgaggtgctgcccagcaccaaccaggagtacatcacctgcaagttcaccaccgtggtgcccagccccaagatcaagtgctgcggcagcctggagtgccagcccgccgcccacgccgactacacctgcaaggtgttcggcggcgtgtaccccttcatgtggggcggcgcccagtgcttctgcgacagcgagaacagccagatgagcgaggcctacgtggagctgagcgccgactgcgccagcgaccacgcccaggccatcaaggtgcacaccgccgccatgaaggtgggcctgagaatcgtgtacggcaacaccaccagcttcctggacgtgtacgtgaacggcgtgacccccggcaccagcaaggacctgaaggtgatcgccggccccatcagcgccagcttcacccccttcgaccacaaggtggtgatccacagaggcctggtgtacaactacgacttccccgagtacggcgccatgaagcccggcgccttcggcgacatccaggccaccagcctgaccagcaaggacctgatcgccagcaccgacatcagactgctgaagcccagcgccaagaacgtgcacgtgccctacacccaggccagcagcggcttcgagatgtggaagaacaacagcggcagacccctgcaggagaccgcccccttcggctgcaagatcgccgtgaaccccctgagagccgtggactgcagctacggcaacatccccatcagcatcgacatccccaacgccgccttcatcagaaccagcgacgcccccctggtgagcaccgtgaagtgcgaggtgagcgagtgcacctacagcgccgacttcggcggcatggccaccctgcagtacgtgagcgacagagagggccagtgccccgtgcacagccacagcagcaccgccaccctgcaggagagcaccgtgcacgtgctggagaagggcgccgtgaccgtgcacttcagcaccgccagcccccaggccaacttcatcgtgagcctgtgcggcaagaagaccacctgcaacgccgagtgcaagccccccgccgaccacatcgtgagcaccccccacaagaacgaccaggagttccaggccgccatcagcaagaccagctggagctggctgttcgccctgttcggcggcgccagcagcctgctgatcatcggcctgatgatcttcgcctgcagcatgatgctgaccagcaccagaagataactcaaatcctgcacaacagattcttcatgtttggaccaaatcaacttgtgataccatgctcaaagaggcctcaattatatttgagtttttaatttttatgaaaaaaaaaaaaaaaaacggaattcaccccaccagtgcaggctgcctatcagaaagtggtggctggtgtggctaatgccctggcccacaagtatcactaagctcgctttcttgctgtccaatttctattaaaggttcctttgttccctaagtccaactactaaactgggggatattatgaagggccttgagcatctggattctgcctaataaaaaacatttattttcattgcaatgatgtatttaaattatttctgaatattttactaaaaagggaatgtgggaggtcagtgcatttaaaacataaagaaatgaagagctagttcaaaccttgggaaaatacactatatcttaaactccatgaaagaaggtgaggctgcaaacagctaatgcacattggcaacagcccctgatgcctatgccttattcatccctcagaaaaggattcaagtagaggcttgatttggaggttaaagttttgctatgctgtattttacattacttattgttttagctgtcctcatgaatgtcttttcactacccatttgcttatcctgcatctctcagccttgactccactcagttctcttgcttagagataccacctttcccctgaagtgttccttccatgttttacggcgagatggtttctcctcgcctggccactcagccttagttgtctctgttgtcttatagaggtctac

SEQ ID NO: 4 - DNA, 7250 bp, synthetic construct
  source 1..7250: mol_type = other DNA
ggatcccctgagggggcccccatgggctagaggatccggcctcggcctctgcataaataaaaaaaattagtcagccatgagcttggcccattgcatacgttgtatccatatcataatatgtacatttatattggctcatgtccaacattaccgccatgttgacattgattattgactagttattaatagtaatcaattacggggtcattagttcatagcccatatatggagttccgcgttacataacttacggtaaatggcccgcctggctgaccgcccaacgacccccgcccattgacgtcaataatgacgtatgttcccatagtaacgccaatagggactttccattgacgtcaatgggtggagtatttacggtaaactgcccacttggcagtacatcaagtgtatcatatgccaagtacgccccctattgacgtcaatgacggtaaatggcccgcctggcattatgcccagtacatgaccttatgggactttcctacttggcagtacatctacgtattagtcatcgctattaccatggtgatgcggttttggcagtacatcaatgggcgtggatagcggtttgactcacggggatttccaagtctccaccccattgacgtcaatgggagtttgttttggcaccaaaatcaacgggactttccaaaatgtcgtaacaactccgccccattgacgcaaatgggcggtaggcgtgtacggtgggaggtctatataagcagagctcgtttagtgaaccgtcagatcgcctggagacgccatccacgctgttttgacctccatagaagacaccgggaccgatccagcctcccctcgaagcttacatgtggtaccgagctcggatcctgagaacttcagggtgagtctatgggacccttgatgttttctttccccttcttttctatggttaagttcatgtcataggaaggggagaagtaacagggtacacatattgaccaaatcagggtaattttgcatttgtaattttaaaaaatgctttcttcttttaatatacttttttgtttatcttatttctaatactttccctaatctctttctttcagggcaataatgatacaatgtatcatgcctctttgcaccattctaaagaataacagtgataatttctgggttaaggcaatagcaatatttctgcatataaatatttctgcatataaattgtaactgatgtaagaggtttcatattgctaatagcagctacaatccagctaccattctgcttttattttatggttgggataaggctggattattctgagtccaagctaggcccttttgctaatcatgttcatacctcttatcttcctcccacagctcctgggcaacgtgctggtctgtgtgctggcccatcactttggcaaagcacgtgagatctgaattctgacactgccaccatgagcgctgctcctctggtgaccgctatgtgcctgctgggaaacgtgtcttttccttgtgacagaccccccacctgctacaccagagagccttctagagccctggacatcctggaggagaacgtgaaccacgaggcttacgacaccctgctgaacgctatcctgcgctgcggaagcagcggatctgtgatcgacgacttcaccctgacctccccctatctgggcacctgtagctattgccaccacaccgtgccctgctttagccctgtgaagattgagcaggtgtgggacgaggccgacgacaataccattagaatccagaccagcgcccagttcggctatgaccagagcggagctgccagcgctaataaataccggtacatggctgccgccgcctacccttatgatgtgcctgactacgccaccgtgaaggagggaaccatggatgacatcaagatcagcacctccggaccttgtagaagactgagctacaaaggctacttcctgctggccaagtgcccccctggagattctgtgaccgtgagtatcgtgagcagcaacagcgccaccagctgcacactggctagaaaaatcaaaccaaaattcgtgggcagagagaagtacgacctgccacccgtgcacggaaagaagatcccctgcacagtgtacgacagactggccgctaccacagccggatacatcaccatgcacagacccaggccccatgcttacaccagctacctggaagaatcctccggcaaagtgtacgccaaaccccccagcggaaaaaacatcacctacgagtgcaagtgcggcgactacaagaccggcaccgtgagcaccagaaccgagatcaccggctgcaccgccatcaagcagtgcgtggcctacaagagcgaccagaccaagtgggtgttcaacagccccgacctgatcagacacgacgaccacaccgcccagggcaagctgcacctgcccttcaagctgatccccagcacctgcatggtgcccgtggcccacgcccccaacgtgatccacggcttcaagcacatcagcctgcagctggacaccgaccacctgaccctgctgaccaccagaagactgggcgccaaccccgagcccaccaccgagtggatcgtgggcaagaccgtgagaaacttcaccgtggacagagacggcctggagtacatctggggcaaccacgagcccgtgagagtgtacgcccaggagagcgcccccggcgacccccacggctggccccacgagatcgtgcagcactactaccacagacaccccgtgtacaccatcctggccgtggccagcgccaccgtggccatgatgatcggcgtgaccgtggccgtgctgtgcgcctgcaaggccagaagagagtgcctgaccccctacgccctggcccccaacgccgtgatccccaccagcctggccctgctgtgctgcgtgagaagcgccaacgccgagaccttcaccgagaccatgagctacctgtggagcaacagccagcccttcttctgggtgcagctgtgcatccccctggccgccttcatcgtgctgatgagatgctgcagctgctgcctgcccttcctggtggtggccggcgcctacctggccaaggtggacgcctacgagcacgccaccaccgtgcccaacgtgccccagatcccctacaaggccctggtggagagagccggctacgcccccctgaacctggagatcaccgtgatgagcagcgaggtgctgcccagcaccaaccaggagtacatcacctgcaagttcaccaccgtggtgcccagccccaagatcaagtgctgcggcagcctggagtgccagcccgccgcccacgccgactacacctgcaaggtgttcggcggcgtgtaccccttcatgtggggcggcgcccagtgcttctgcgacagcgagaacagccagatgagcgaggcctacgtggagctgagcgccgactgcgccagcgaccacgcccaggccatcaaggtgcacaccgccgccatgaaggtgggcctgagaatcgtgtacggcaacaccaccagcttcctggacgtgtacgtgaacggcgtgacccccggcaccagcaaggacctgaaggtgatcgccggccccatcagcgccagcttcacccccttcgaccacaaggtggtgatccacagaggcctggtgtacaactacgacttccccgagtacggcgccatgaagcccggcgccttcggcgacatccaggccaccagcctgaccagcaaggacctgatcgccagcaccgacatcagactgctgaagcccagcgccaagaacgtgcacgtgccctacacccaggccagcagcggcttcgagatgtggaagaacaacagcggcagacccctgcaggagaccgcccccttcggctgcaagatcgccgtgaaccccctgagagccgtggactgcagctacggcaacatccccatcagcatcgacatccccaacgccgccttcatcagaaccagcgacgcccccctggtgagcaccgtgaagtgcgaggtgagcgagtgcacctacagcgccgacttcggcggcatggccaccctgcagtacgtgagcgacagagagggccagtgccccgtgcacagccacagcagcaccgccaccctgcaggagagcaccgtgcacgtgctggagaagggcgccgtgaccgtgcacttcagcaccgccagcccccaggccaacttcatcgtgagcctgtgcggcaagaagaccacctgcaacgccgagtgcaagccccccgccgaccacatcgtgagcaccccccacaagaacgaccaggagttccaggccgccatcagcaagaccagctggagctggctgttcgccctgttcggcggcgccagcagcctgctgatcatcggcctgatgatcttcgcctgcagcatgatgctgaccagcaccagaagataactcaaatcctgcacaacagattcttcatgtttggaccaaatcaacttgtgataccatgctcaaagaggcctcaattatatttgagtttttaatttttatgaaaaaaaaaaaaaaaaacggaattcaccccaccagtgcaggctgcctatcagaaagtggtggctggtgtggctaatgccctggcccacaagtatcactaagctcgctttcttgctgtccaatttctattaaaggttcctttgttccctaagtccaactactaaactgggggatattatgaagggccttgagcatctggattctgcctaataaaaaacatttattttcattgcaatgatgtatttaaattatttctgaatattttactaaaaagggaatgtgggaggtcagtgcatttaaaacataaagaaatgaagagctagttcaaaccttgggaaaatacactatatcttaaactccatgaaagaaggtgaggctgcaaacagctaatgcacattggcaacagcccctgatgcctatgccttattcatccctcagaaaaggattcaagtagaggcttgatttggaggttaaagttttgctatgctgtattttacattacttattgttttagctgtcctcatgaatgtcttttcactacccatttgcttatcctgcatctctcagccttgactccactcagttctcttgcttagagataccacctttcccctgaagtgttccttccatgttttacggcgagatggtttctcctcgcctggccactcagccttagttgtctctgttgtcttatagaggtctacttgaagaaggaaaaacagggggcatggtttgactgtcctgtgagcccttcttccctgcctcccccactcacagtgacccggaatccctcgacatggcagtctagcactagtgcggccgcagatctgcttcctcgctcactgactcgctgcgctcggtcgttcggctgcggcgagcggtatcagctcactcaaaggcggtaatacggttatccacagaatcaggggataacgcaggaaagaacatgtgagcaaaaggccagcaaaaggccaggaaccgtaaaaaggccgcgttgctggcgtttttccataggctccgcccccctgacgagcatcacaaaaatcgacgctcaagtcagaggtggcgaaacccgacaggactataaagataccaggcgtttccccctggaagctccctcgtgcgctctcctgttccgaccctgccgcttaccggatacctgtccgcctttctcccttcgggaagcgtggcgctttctcatagctcacgctgtaggtatctcagttcggtgtaggtcgttcgctccaagctgggctgtgtgcacgaaccccccgttcagcccgaccgctgcgccttatccggtaactatcgtcttgagtccaacccggtaagacacgacttatcgccactggcagcagccactggtaacaggattagcagagcgaggtatgtaggcggtgctacagagttcttgaagtggtggcctaactacggctacactagaagaacagtatttggtatctgcgctctgctgaagccagttaccttcggaaaaagagttggtagctcttgatccggcaaacaaaccaccgctggtagcggtggtttttttgtttgcaagcagcagattacgcgcagaaaaaaaggatctcaagaagatcctttgatcttttctacggggtctgacgctcagtggaacgaaaactcacgttaagggattttggtcatgagattatcaaaaaggatcttcacctagatccttttaaattaaaaatgaagttttaaatcaatctaaagtatatatgagtaaacttggtctgacagttaccaatgcttaatcagtgaggcacctatctcagcgatctgtctatttcgttcatccatagttgcctgactccccgtcgtgtagataactacgatacgggagggcttaccatctggccccagtgctgcaatgataccgcgagacccacgctcaccggctccagatttatcagcaataaaccagccagccggaagggccgagcgcagaagtggtcctgcaactttatccgcctccatccagtctattaattgttgccgggaagctagagtaagtagttcgccagttaatagtttgcgcaacgttgttgccattgctacaggcatcgtggtgtcacgctcgtcgtttggtatggcttcattcagctccggttcccaacgatcaaggcgagttacatgatcccccatgttgtgcaaaaaagcggttagctccttcggtcctccgatcgttgtcagaagtaagttggccgcagtgttatcactcatggttatggcagcactgcataattctcttactgtcatgccatccgtaagatgcttttctgtgactggtgagtactcaaccaagtcattctgagaatagtgtatgcggcgaccgagttgctcttgcccggcgtcaatacgggataataccgcgccacatagcagaactttaaaagtgctcatcattggaaaacgttcttcggggcgaaaactctcaaggatcttaccgctgttgagatccagttcgatgtaacccactcgtgcacccaactgatcttcagcatcttttactttcaccagcgtttctgggtgagcaaaaacaggaaggcaaaatgccgcaaaaaagggaataagggcgacacggaaatgttgaatactcatactcttcctttttcaatattattgaagcatttatcagggttattgtctcatgagcggatacatatttgaatgtatttagaaaaataaacaaataggggttccgcgcacatttccccgaaaagtgccacctgacgt

SEQ ID NO: 5 - DNA, 4174 bp, synthetic construct
  source 1..4174: mol_type = other DNA
agcgcccaatacgcaaaccgcctctccccgcgcgttggccgattcattaatgcagctggcacgacaggtttcccgactggaaagcgggcagtgagcgcaacgcaattaatgtgagttagctcactcattaggcaccccaggctttacactttatgcttccggctcgtatgttgtgtggaattgtgagcggataacaatttcacacaggaaacagctatgaccatgattacgaattcgatgtacgggccagatatacgcgtatctgaggggactaggtgtgtttaggcgaaaagcggggcttcggttgtacgcggttaggagtcccctcaggattagtagtttcgcttttgcatagggagggggaaatgtagtcttatgcaatacacttgtagtcttgcaacatggtaacgatgagttagcaacatgccttacaaggagagaaaaagcaccgtgcatgccgattggtggaagtaaggtggtacgatcgtgccttattaggaaggcaacagacaggtctgacatggattggacgaaccactgaattccgcattgcagagataattgtatttaagtgcctagctcgatacaataaacgccatttgaccattcaccacattggtgtgcacctccaagctcgagctcgtttagtgaaccgtcagatcgcctggagacgccatccacgctgttttgacctccatagaagacaccgggaccgatccagcctcccctcgaagctagtcgattaggcatctcctatggcaggaagaagcggagacagcgacgaagacctcctcaaggcagtcagactcatcaagtttctctatcaaagcaacccacctcccaatcccgaggggacccgacaggcccgaaggaatagaagaagaaggtggagagagagacagagacagatccattcgattagtgaacggatccttagcacttatctgggacgatctgcggagcctgtgcctcttcagctaccaccgcttgagagacttactcttgattgtaacgaggattgtggaacttctgggacgcagggggtgggaagccctcaaatattggtggaatctcctacaatattggagtcaggagctaaagaatagtgctgttagcttgctcaatgccacagctatagcagtagctgaggggacagatagggttatagaagtagtacaagaagcttggcactggccgtcgttttacatgatctgagcctgggagatctctggctaactagggaacccactgcttaagcctcaataaagcttgccttgagtgcttcaagtagtgtgtgcccgtctgttgtgtgactctggtaactagagatcaggaaaaccctggcgttacccaacttaatcgccttgcagcacatccccctttcgccagctggcgtaatagcgaagaggcccgcaccgatcgcccttcccaacagttgcgcagcctgaatggcgaatggcgcctgatgcggtattttctccttacgcatctgtgcggtatttcacaccgcatacgtcaaagcaaccatagtacgcgccctgtagcggcgcattaagcgcggcgggtgtggtggttacgcgcagcgtgaccgctacacttgccagcgccctagcgcccgctcctttcgctttcttcccttcctttctcgccacgttcgccggctttccccgtcaagctctaaatcgggggctccctttagggttccgatttagtgctttacggcacctcgaccccaaaaaacttgatttgggtgatggttcacgtagtgggccatcgccctgatagacggtttttcgccctttgacgttggagtccacgttctttaatagtggactcttgttccaaactggaacaacactcaaccctatctcgggctattcttttgatttataagggattttgccgatttcggcctattggttaaaaaatgagctgatttaacaaaaatttaacgcgaattttaacaaaatattaacgtttacaattttatggtgcactctcagtacaatctgctctgatgccgcatagttaagccagccccgacacccgccaacacccgctgacgcgccctgacgggcttgtctgctcccggcatccgcttacagacaagctgtgaccgtctccgggagctgcatgtgtcagaggttttcaccgtcatcaccgaaacgcgcgagacgaaagggcctcgtgatacgcctatttttataggttaatgtcatgataataatggtttcttagacgtcaggtggcacttttcggggaaatgtgcgcggaacccctatttgtttatttttctaaatacattcaaatatgtatccgctcatgagacaataaccctgataaatgcttcaataatattgaaaaaggaagagtatgagtattcaacatttccgtgtcgcccttattcccttttttgcggcattttgccttcctgtttttgctcacccagaaacgctggtgaaagtaaaagatgctgaagatcagttgggtgcacgagtgggttacatcgaactggatctcaacagcggtaagatccttgagagttttcgccccgaagaacgttttccaatgatgagcacttttaaagttctgctatgtggcgcggtattatcccgtattgacgccgggcaagagcaactcggtcgccgcatacactattctcagaatgacttggttgagtactcaccagtcacagaaaagcatcttacggatggcatgacagtaagagaattatgcagtgctgccataaccatgagtgataacactgcggccaacttacttctgacaacgatcggaggaccgaaggagctaaccgcttttttgcacaacatgggggatcatgtaactcgccttgatcgttgggaaccggagctgaatgaagccataccaaacgacgagcgtgacaccacgatgcctgtagcaatggcaacaacgttgcgcaaactattaactggcgaactacttactctagcttcccggcaacaattaatagactggatggaggcggataaagttgcaggaccacttctgcgctcggcccttccggctggctggtttattgctgataaatctggagccggtgagcgtgggtctcgcggtatcattgcagcactggggccagatggtaagccctcccgtatcgtagttatctacacgacggggagtcaggcaactatggatgaacgaaatagacagatcgctgagataggtgcctcactgattaagcattggtaactgtcagaccaagtttactcatatatactttagattgatttaaaacttcatttttaatttaaaaggatctaggtgaagatcctttttgataatctcatgaccaaaatcccttaacgtgagttttcgttccactgagcgtcagaccccgtagaaaagatcaaaggatcttcttgagatcctttttttctgcgcgtaatctgctgcttgcaaacaaaaaaaccaccgctaccagcggtggtttgtttgccggatcaagagctaccaactctttttccgaaggtaactggcttcagcagagcgcagataccaaatactgtccttctagtgtagccgtagttaggccaccacttcaagaactctgtagcaccgcctacatacctcgctctgctaatcctgttaccagtggctgctgccagtggcgataagtcgtgtcttaccgggttggactcaagacgatagttaccggataaggcgcagcggtcgggctgaacggggggttcgtgcacacagcccagcttggagcgaacgacctacaccgaactgagatacctacagcgtgagctatgagaaagcgccacgcttcccgaagggagaaaggcggacaggtatccggtaagcggcagggtcggaacaggagagcgcacgagggagcttccagggggaaacgcctggtatctttatagtcctgtcgggtttcgccacctctgacttgagcgtcgatttttgtgatgctcgtcaggggggcggagcctatggaaaaacgccagcaacgcggcctttttacggttcctggccttttgctggccttttgctcacatgttctttcctgcgttatcccctgattctgtggataaccgtattaccgcctttgagtgagctgataccgctcgccgcagccgaacgaccgagcgcagcgagtcagtgagcgaggaagcggaag

SEQ ID NO: 6 - DNA, 7910 bp, synthetic construct
  source 1..7910: mol_type = other DNA
tcgcgcgtttcggtgatgacggtgaaaacctctgacacatgcagctcccggagacggtcacagcttgtctgtaagcggatgccgggagcagacaagcccgtcagggcgcgtcagcgggtgttggcgggtgtcggggctggcttaactatgcggcatcagagcagattgtactgagagtgcaccatatgcggtgtgaaataccgcacagatgcgtaaggagaaaataccgcatcaggcgccattcgccattcaggctgcgcaactgttgggaagggcgatcggtgcgggcctcttcgctattacgccagctggcgaaagggggatgtgctgcaaggcgattaagttgggtaacgccagggttttcccagtcacgacgttgtaaaacgacggccagtgaattcgagcttgcatgcctgcaggtcgttacataacttacggtaaatggcccgcctggctgaccgcccaacgacccccgcccattgacgtcaataatgacgtatgttcccatagtaacgccaatagggactttccattgacgtcaatgggtggactatttacggtaaactgcccacttggcagtacatcaagtgtatcatatgccaagtacgccccctattgacgtcaatgacggtaaatggcccgcctggcattatgcccagtacatgaccttatgggactttcctacttggcagtacatctacgtattagtcatcgctattaccatggtgatgcggttttggcagtacatcaatgggcgtggatagcggtttgactcacggggatttccaagtctccaccccattgacgtcaatgggagtttgttttggcaccaaaatcaacgggactttccaaaatgtcgtaacaactccgccccattgacgcaaatgggcggtaggcgtgtacggtgggaggtctatataagcagagctcgtttagtgaaccgtcagatcgcctggagacgccatccacgctgttttgacctccatagaagacaccgggaccgatccagcctccggactctagaggatccggtactcgaggaactgaaaaaccagaaagttaactggtaagtttagtctttttgtcttttatttcaggtcccgatccggtggtggtgcaaatcaaagaactgctcctcagtggatgttgcctttacttctaggcctgtacggaagtgttacttctgctctaaaagctgcggaattgtacccgcggacgcgtgccaccatggactggacctggatcctgttcctggtggccgccgccacccgcgtgcacagctttgtgtttctggtgctgctgccactggtgagcagccagtgtgtgaatctgaccacacgcacccagctgccacccgcctacacaaatagcttcacaagaggcgtgtactaccctgataaagtgtttaggtctagtgtgctgcactctacccaggatctgttcctgcccttctttagtaatgtgacctggttccacgccatccatgtgagcggaactaacggcactaagagatttgacaacccagtgctgccttttaacgacggagtgtacttcgcctccaccgaaaagtctaatattattaggggatggatcttcgggacaaccctcgacagtaagacccagagcctgctgattgtgaataatgctacaaacgtggtcatcaaggtgtgcgagttccagttttgtaatgatcctttcttgggagtgtactaccacaagaataataagtcatggatggagagtgagtttagggtgtatagttccgccaataactgtacctttgaatacgtgagtcagccctttctgatggacctggaaggaaaacagggcaattttaagaatctgcgcgaatttgtgtttaaaaatatcgacggctatttcaaaatctacagcaagcacacccccatcaacctggtgagagacctgccccagggcttcagcgccctggagcccctggtggatctccccatcgggatcaatatcacacggttccagacactgctggccctgcacagaagctatctgacacctggagactcctcctccggctggaccgccggcgcagccgcatactatgtgggctacctgcagccaaggaccttcctgctgaaatataacgagaacggaaccattacagatgccgtggattgtgccctggatcccctgtctgagaccaaatgcaccctgaaaagttttaccgtggagaagggcatctatcagaccagcaatttccgggtgcagcccactgagtccatcgtccggtttcctaatattaccaacctgtgccccttcggcgaggtctttaatgctacaagattcgccagcgtgtacgcctggaatagaaaaagaatttccaactgtgtcgccgactattccgtgctgtataacagtgccagcttctccaccttcaaatgttacggagtgagccccacaaagctgaacgacctgtgcttcaccaacgtctacgccgatagcttcgtgattagaggcgacgaagtccggcagattgctccaggccagaccggaaagattgccgattacaactataaactccctgatgactttaccggatgcgtgattgcttggaacagtaacaacctggatagcaaagtgggcgggaattataactacctgtaccggctcttcagaaaatctaatttgaaacccttcgagcgggacatcagcactgagatctaccaggccggctctaccccctgtaacggagtggagggcttcaactgctatttcccactgcagagctatggattccagcccactaacggcgtcggatatcagccatatagggtggtggtgctgtccttcgaactcctccacgcccccgctaccgtgtgcggccctaagaagtctacaaacctggttaaaaataagtgcgtgaactttaactttaacggcctgacaggcactggcgttctgacagaatctaacaagaagttcctgcccttccagcagttcggccgggacatcgctgacaccaccgacgccgtgagggacccccagacactggagatccttgacatcactccttgctccttcggcggcgtgtctgtgatcacacccggcacaaacactagtaaccaggtggcagttctgtaccaggatgtgaactgcactgaggtccccgttgcaatccacgccgatcagctgacccccacttggcgcgtgtactcaaccggcagtaatgtgttccagacccgcgccggctgcctgataggagccgagcacgtcaataatagttacgagtgtgatatccctattggtgccggaatctgtgcttcataccagacccagaccaattcacccaggcgagcacgctccgtcgcttcccagagtattatcgcctacactatgtccctcggggcagaaaacagcgtcgcctatagcaacaatagcatcgctattccaacaaacttcaccatctccgtgaccacagagattctgcccgtgtccatgactaagacatccgtggattgcaccatgtatatttgtggtgactctaccgagtgctctaacctcctgctgcagtacggctctttctgcacacagctcaatcgcgcactgaccgggatcgctgtggagcaggacaagaacactcaggaagtgttcgcacaggtgaagcagatctataagacccctcccatcaaagatttcggaggattcaatttctcacagatcctgcccgacccaagcaagccatctaaacgctctttcattgaggatctgctgttcaataaggtgaccctggctgatgccgggttcatcaagcagtatggcgactgcctcggcgatatcgctgccagggacctgatctgcgcacagaaattcaatggactgaccgtcctgccaccactgctgacagatgagatgatcgcccagtatacttctgccctgctcgccggcaccatcacttctgggtggacctttggcgccggcgcagccctgcagatccctttcgccatgcagatggcttaccgctttaatggaatcggggtgacccagaacgtgctgtatgagaatcagaaactgattgcaaatcagtttaacagcgctatcggcaaaatccaggattctctgagctccacagccagcgccctcggaaagctgcaggatgtcgtgaaccagaatgcccaggcgctgaataccctggtgaaacagctcagctctaacttcggcgctatttcctccgtgctcaacgatatcctgagcaggctggatcctcccgaagccgaagtgcagattgacagactgatcacaggcaggctccagagcctccagacatacgtcacccagcagctgattcgggctgccgagatacgggcaagcgctaacctggccgccactaagatgagcgagtgtgtgctcggccagagcaagcgggtggacttttgcgggaaaggctatcacctgatgtctttcccacagtccgcccctcacggggttgtgttcctgcacgtgacctacgtgcccgcccaggagaagaatttcacaaccgcacccgccatctgccatgacgggaaagcccactttcccagggagggcgtgttcgtgagcaatggcactcactggtttgtgacccagagaaatttctatgagccccagatcatcaccaccgacaatacctttgtcagtggcaactgtgatgtcgtgattggcatcgtgaacaacactgtgtacgatcctctgcagcccgagctggactcctttaaagaggagctggacaagtatttcaaaaaccacacatccccagatgtggatctgggcgatatctccggcatcaacgccagtgtggtgaatatccagaaagagattgatagactgaacgaggtggctaagaacctgaacgaatccctgattgacctgcaggagctgggaaagtacgagcagtatattaagtggccttggtatatctggctggggttcatcgctggactgatcgctattgtgatggtgaccattatgctgtgctgcatgactagctgctgtagttgcctgaagggatgctgtagctgcggcagctgctgcaagtttgatgaggacgattctgagcctgtgctgaaaggggtgaagctgcactacaccgattacaaagacgatgacgataagtaaaccggtcttgcagcacatacatgaggatcacccatgtctgcaggtcgactctagaaaacatgaggatcacccatgtctgcagtattcccgggttcattagatcctaaggtacctaattgcctagaaaacatgaggatcacccatgtctgcaggtcgactctagaaaacatgaggatcacccatgtctgcagtattcccgggttcattagatcctaaggtacctaattgcctagaaaacatgaggatcacccatgtctgcaggtcgactctagaaaacatgaggatcacccatgtgtgcaccttaagcttggcccgcggggatccagacatgataagatacattgatgagtttggacaaaccacaactagaatgcagtgaaaaaaatgctttatttgtgaaatttgtgatgctattgctttatttgtaaccattataagctgcaataaacaagttaacaacaacaattgcattcattttatgtttcaggttcagggggaggtgtgggaggttttttcggatcctctagagtcgacctgcaggcatgcaagcttggcgtaatcatggtcatagctgtttcctgtgtgaaattgttatccgctcacaattccacacaacatacgagccggaagcataaagtgtaaagcctggggtgcctaatgagtgagctaactcacattaattgcgttgcgctcactgcccgctttccagtcgggaaacctgtcgtgccagctgcattaatgaatcggccaacgcgcggggagaggcggtttgcgtattgggcgctcttccgcttcctcgctcactgactcgctgcgctcggtcgttcggctgcggcgagcggtatcagctcactcaaaggcggtaatacggttatccacagaatcaggggataacgcaggaaagaacatgtgagcaaaaggccagcaaaaggccaggaaccgtaaaaaggccgcgttgctggcgtttttccataggctccgcccccctgacgagcatcacaaaaatcgacgctcaagtcagaggtggcgaaacccgacaggactataaagataccaggcgtttccccctggaagctccctcgtgcgctctcctgttccgaccctgccgcttaccggatacctgtccgcctttctcccttcgggaagcgtggcgctttctcatagctcacgctgtaggtatctcagttcggtgtaggtcgttcgctccaagctgggctgtgtgcacgaaccccccgttcagcccgaccgctgcgccttatccggtaactatcgtcttgagtccaacccggtaagacacgacttatcgccactggcagcagccactggtaacaggattagcagagcgaggtatgtaggcggtgctacagagttcttgaagtggtggcctaactacggctacactagaaggacagtatttggtatctgcgctctgctgaagccagttaccttcggaaaaagagttggtagctcttgatccggcaaacaaaccaccgctggtagcggtggtttttttgtttgcaagcagcagattacgcgcagaaaaaaaggatctcaagaagatcctttgatcttttctacggggtctgacgctcagtggaacgaaaactcacgttaagggattttggtcatgagattatcaaaaaggatcttcacctagatccttttaaattaaaaatgaagttttaaatcaatctaaagtatatatgagtaaacttggtctgacagttaccaatgcttaatcagtgaggcacctatctcagcgatctgtctatttcgttcatccatagttgcctgactccccgtcgtgtagataactacgatacgggagggcttaccatctggccccagtgctgcaatgataccgcgagacccacgctcaccggctccagatttatcagcaataaaccagccagccggaagggccgagcgcagaagtggtcctgcaactttatccgcctccatccagtctattaattgttgccgggaagctagagtaagtagttcgccagttaatagtttgcgcaacgttgttgccattgctacaggcatcgtggtgtcacgctcgtcgtttggtatggcttcattcagctccggttcccaacgatcaaggcgagttacatgatcccccatgttgtgcaaaaaagcggttagctccttcggtcctccgatcgttgtcagaagtaagttggccgcagtgttatcactcatggttatggcagcactgcataattctcttactgtcatgccatccgtaagatgcttttctgtgactggtgagtactcaaccaagtcattctgagaatagtgtatgcggcgaccgagttgctcttgcccggcgtcaatacgggataataccgcgccacatagcagaactttaaaagtgctcatcattggaaaacgttcttcggggcgaaaactctcaaggatcttaccgctgttgagatccagttcgatgtaacccactcgtgcacccaactgatcttcagcatcttttactttcaccagcgtttctgggtgagcaaaaacaggaaggcaaaatgccgcaaaaaagggaataagggcgacacggaaatgttgaatactcatactcttcctttttcaatattattgaagcatttatcagggttattgtctcatgagcggatacatatttgaatgtatttagaaaaataaacaaataggggttccgcgcacatttccccgaaaagtgccacctgacgtctaagaaaccattattatcatgacattaacctataaaaataggcgtatcacgaggccctttcgtc

SEQ ID NO: 7 - DNA, 8895 bp, synthetic construct
  source 1..8895: mol_type = other DNA
ggatcccctgagggggcccccatgggctagaggatccggcctcggcctctgcataaataaaaaaaattagtcagccatgagcttggcccattgcatacgttgtatccatatcataatatgtacatttatattggctcatgtccaacattaccgccatgttgacattgattattgactagttattaatagtaatcaattacggggtcattagttcatagcccatatatggagttccgcgttacataacttacggtaaatggcccgcctggctgaccgcccaacgacccccgcccattgacgtcaataatgacgtatgttcccatagtaacgccaatagggactttccattgacgtcaatgggtggagtatttacggtaaactgcccacttggcagtacatcaagtgtatcatatgccaagtacgccccctattgacgtcaatgacggtaaatggcccgcctggcattatgcccagtacatgaccttatgggactttcctacttggcagtacatctacgtattagtcatcgctattaccatggtgatgcggttttggcagtacatcaatgggcgtggatagcggtttgactcacggggatttccaagtctccaccccattgacgtcaatgggagtttgttttggcaccaaaatcaacgggactttccaaaatgtcgtaacaactccgccccattgacgcaaatgggcggtaggcgtgtacggtgggaggtctatataagcagagctcgtttagtgaaccgtcagatcgcctggagacgccatccacgctgttttgacctccatagaagacaccgggaccgatccagcctcccctcgaagcttacatgtggtaccgagctcggatcctgagaacttcagggtgagtctatgggacccttgatgttttctttccccttcttttctatggttaagttcatgtcataggaaggggagaagtaacagggtacacatattgaccaaatcagggtaattttgcatttgtaattttaaaaaatgctttcttcttttaatatacttttttgtttatcttatttctaatactttccctaatctctttctttcagggcaataatgatacaatgtatcatgcctctttgcaccattctaaagaataacagtgataatttctgggttaaggcaatagcaatatttctgcatataaatatttctgcatataaattgtaactgatgtaagaggtttcatattgctaatagcagctacaatccagctaccattctgcttttattttatggttgggataaggctggattattctgagtccaagctaggcccttttgctaatcatgttcatacctcttatcttcctcccacagctcctgggcaacgtgctggtctgtgtgctggcccatcactttggcaaagcacgtgagatctgaattcgagatctgccgccgccatgggtgcgagagcgtcagtattaagcgggggagaattagatcgatgggaaaaaattcggttaaggccagggggaaagaaaaaatataaattaaaacatatagtatgggcaagcagggagctagaacgattcgcagttaatcctggcctgttagaaacatcagaaggctgtagacaaatactgggacagctacaaccatcccttcagacaggatcagaagaacttagatcattatataatacagtagcaaccctctattgtgtgcatcaaaggatagagataaaagacaccaaggaagctttagacaagatagaggaagagcaaaacaaaagtaagaaaaaagcacagcaagcagcagctgacacaggacacagcaatcaggtcagccaaaattaccctatagtgcagaacatccaggggcaaatggtacatcaggccatatcacctagaactttaaatgcatgggtaaaagtagtagaagagaaggctttcagcccagaagtgatacccatgttttcagcattatcagaaggagccaccccacaagatttaaacaccatgctaaacacagtggggggacatcaagcagccatgcaaatgttaaaagagaccatcaatgaggaagctgcagaatgggatagagtgcatccagtgcatgcagggcctattgcaccaggccagatgagagaaccaaggggaagtgacatagcaggaactactagtactagtacccttcaggaacaaataggatggatgacacataatccacctatcccagtaggagaaatctataaaagatggataatcctgggattaaataaaatagtaagaatgtatagccctaccagcattctggacataagacaaggaccaaaggaaccctttagagactatgtagaccgattctataaaactctaagagccgagcaagcttcacaagaggtaaaaaattggatgacagaaaccttgttggtccaaaatgcgaacccagattgtaagactattttaaaagcattgggaccaggagcgacactagaagaaatgatgacagcatgtcagggagtggggggacccggccataaagcaagagttttggctgaagcaatgagccaagtaacaaatccagctaccataatgatacagaaaggcaattttaggaaccaaagaaagactgttaagtgtttcaattgtggcaaagaagggcacatagccaaaaattgcagggcccctaggaaaaagggctgttggaaatgtggaaaggaaggacaccaaatgaaagattgtactgagagacaggctaattttttagggaagatctggccttcccacaagggaaggccagggaattttcttcagagcagaccagagccaacagccccaccagaagagagcttcaggtttggggaagagacaacaactccctctcagaagcaggagccgatagacaaggaactgtatcctttagcttccctcagatcactctttggcagcgacccctcgtcacaataaagataggggggcaattaaaggaagctctattagatacaggagcagatgatacagtattagaagaaatgaatttgccaggaagatggaaaccaaaaatgatagggggaattggaggttttatcaaagtaggacagtatgatcagatactcatagaaatctgtggacataaagctataggtacagtattagtaggacctacacctgtcaacataattggaagaaatctgttgactcagattggttgcactttaaattttcccattagccctattgagactgtaccagtaaaattaaagccaggaatggatggcccaaaagttaaacaatggccattgacagaagaaaaaataaaagcattagtagaaatttgtacagagatggaaaaggaagggaaaatttcaaaaattgggcctgaaaatccatacaatactccagtatttgccataaagaaaaaagacagtactaaatggagaaaattagtagatttcagagaacttaataagagaactcaagacttctgggaagttcaattaggaataccacatcccgcagggttaaaaaagaaaaaatcagtaacagtactggatgtgggtgatgcatatttttcagttcccttagatgaagacttcaggaagtatactgcatttaccatacctagtataaacaatgagacaccagggattagatatcagtacaatgtgcttccacagggatggaaaggatcaccagcaatattccaaagtagcatgacaaaaatcttagagccttttagaaaacaaaatccagacatagttatctatcaatacatggatgatttgtatgtaggatctgacttagaaatagggcagcatagaacaaaaatagaggagctgagacaacatctgttgaggtggggacttaccacaccagacaaaaaacatcagaaagaacctccattcctttggatgggttatgaactccatcctgataaatggacagtacagcctatagtgctgccagaaaaagacagctggactgtcaatgacatacagaagttagtggggaaattgaattgggcaagtcagatttacccagggattaaagtaaggcaattatgtaaactccttagaggaaccaaagcactaacagaagtaataccactaacagaagaagcagagctagaactggcagaaaacagagagattctaaaagaaccagtacatggagtgtattatgacccatcaaaagacttaatagcagaaatacagaagcaggggcaaggccaatggacatatcaaatttatcaagagccatttaaaaatctgaaaacaggaaaatatgcaagaatgaggggtgcccacactaatgatgtaaaacaattaacagaggcagtgcaaaaaataaccacagaaagcatagtaatatggggaaagactcctaaatttaaactgcccatacaaaaggaaacatgggaaacatggtggacagagtattggcaagccacctggattcctgagtgggagtttgttaatacccctcccttagtgaaattatggtaccagttagagaaagaacccatagtaggagcagaaaccttctatgtagatggggcagctaacagggagactaaattaggaaaagcaggatatgttactaatagaggaagacaaaaagttgtcaccctaactgacacaacaaatcagaagactgagttacaagcaatttatctagctttgcaggattcgggattagaagtaaacatagtaacagactcacaatatgcattaggaatcattcaagcacaaccagatcaaagtgaatcagagttagtcaatcaaataatagagcagttaataaaaaaggaaaaggtctatctggcatgggtaccagcacacaaaggaattggaggaaatgaacaagtagataaattagtcagtgctggaatcaggaaagtactatttttagatggaatagataaggcccaagatgaacatgagaaatatcacagtaattggagagcaatggctagtgattttaacctgccacctgtagtagcaaaagaaatagtagccagctgtgataaatgtcagctaaaaggagaagccatgcatggacaagtagactgtagtccaggaatatggcaactagtttgtacacatttagaaggaaaagttatcctggtagcagttcatgtagccagtggatatatagaagcagaagttattccagcagaaacagggcaggaaacagcatattttcttttaaaattagcaggaagatggccagtaaaaacaatacatactgacaatggcagcaatttcaccggtgctacggttagggccgcctgttggtgggcgggaatcaagcaggaatttggaattccctacaatccccaaagtcaaggagtagtagaatctatgaataaagaattaaagaaaattataggacaggtaagagatcaggctgaacatcttaagacagcagtacaaatggcagtattcatccacaattttaaaagaaaaggggggattggggggtacagtgcaggggaaagaatagtagacataatagcaacagacatacaaactaaagaattacaaaaacaaattacaaaaattcaaaattttcgggtttattacagggacagcagagatccagtttggaaaggaccagcaaagctcctctggaaaggtgaaggggcagtagtaatacaagataatagtgacataaaagtagtgccaagaagaaaagcaaagatcatcagggattatggaaaacagatggcaggtgatgattgtgtggcaagtagacaggatgaggattaacacatggaattccggagcggccgcaggagctttgttccttgggttcttgggagcagcaggaagcactatgggcgcagcctcaatgacgctgacggtacaggccagacaattattgtctggtatagtgcagcagcagaacaatttgctgagggctattgaggcgcaacagcatctgttgcaactcacagtctggggcatcaagcagctccaggcaagaatcctggctgtggaaagatacctaaaggatcaacagctcctggggatttggggttgctctggaaaactcatttgcaccactgctgtgccttggaatgctagttggagtaataaatctctggaacagatttggaatcacacgacctggatggagtgggacagagaaattaacaattacacaagcttccgcggaattcaccccaccagtgcaggctgcctatcagaaagtggtggctggtgtggctaatgccctggcccacaagtttcactaagctcgcttccttgctgtccaatttctattaaaggttccttggttccctaagtccaactactaaactgggggatattatgaagggccttgagcatctggattctgcctaataaaaaacatttattttcattgcaatgatgtatttaaattatttctgaatattttactaaaaagggaatgtgggaggtcagtgcatttaaaacataaagaaatgaagagctagttcaaaccttgggaaaatacactatatcttaaactccatgaaagaaggtgaggctgcaaacagctaatgcacattggcaacagccctgatgcctatgccttattcatccctcagaaaaggattcaagtagaggcttgatttggaggttaaagtttggctatgctgtattttacattacttattgttttagctgtcctcatgaatgtcttttcactacccatttgcttatcctgcatctctcagccttgactccactcagttctcttgcttagagataccacctttcccctgaagtgttccttccatgttttacggcgagatggtttctcctcgcctggccactcagccttagttgtctctgttgtcttatagaggtctacttgaagaaggaaaaacagggggcatggtttgactgtcctgtgagcccttcttccctgcctcccccactcacagtgacccggaatccctcgacatggcagtctagcactagtgcggccgcagatctgcttcctcgctcactgactcgctgcgctcggtcgttcggctgcggcgagcggtatcagctcactcaaaggcggtaatacggttatccacagaatcaggggataacgcaggaaagaacatgtgagcaaaaggccagcaaaaggccaggaaccgtaaaaaggccgcgttgctggcgtttttccataggctccgcccccctgacgagcatcacaaaaatcgacgctcaagtcagaggtggcgaaacccgacaggactataaagataccaggcgtttccccctggaagctccctcgtgcgctctcctgttccgaccctgccgcttaccggatacctgtccgcctttctcccttcgggaagcgtggcgctttctcaatgctcacgctgtaggtatctcagttcggtgtaggtcgttcgctccaagctgggctgtgtgcacgaaccccccgttcagcccgaccgctgcgccttatccggtaactatcgtcttgagtccaacccggtaagacacgacttatcgccactggcagcagccactggtaacaggattagcagagcgaggtatgtaggcggtgctacagagttcttgaagtggtggcctaactacggctacactagaaggacagtatttggtatctgcgctctgctgaagccagttaccttcggaaaaagagttggtagctcttgatccggcaaacaaaccaccgctggtagcggtggtttttttgtttgcaagcagcagattacgcgcagaaaaaaaggatctcaagaagatcctttgatcttttctacggggtctgacgctcagtggaacgaaaactcacgttaagggattttggtcatgagattatcaaaaaggatcttcacctagatccttttaaattaaaaatgaagttttaaatcaatctaaagtatatatgagtaaacttggtctgacagttaccaatgcttaatcagtgaggcacctatctcagcgatctgtctatttcgttcatccatagttgcctgactccccgtcgtgtagataactacgatacgggagggcttaccatctggccccagtgctgcaatgataccgcgagacccacgctcaccggctccagatttatcagcaataaaccagccagccggaagggccgagcgcagaagtggtcctgcaactttatccgcctccatccagtctattaattgttgccgggaagctagagtaagtagttcgccagttaatagtttgcgcaacgttgttgccattgctacaggcatcgtggtgtcacgctcgtcgtttggtatggcttcattcagctccggttcccaacgatcaaggcgagttacatgatcccccatgttgtgcaaaaaagcggttagctccttcggtcctccgatcgttgtcagaagtaagttggccgcagtgttatcactcatggttatggcagcactgcataattctcttactgtcatgccatccgtaagatgcttttctgtgactggtgagtactcaaccaagtcattctgagaatagtgtatgcggcgaccgagttgctcttgcccggcgtcaatacgggataataccgcgccacatagcagaactttaaaagtgctcatcattggaaaacgttcttcggggcgaaaactctcaaggatcttaccgctgttgagatccagttcgatgtaacccactcgtgcacccaactgatcttcagcatcttttactttcaccagcgtttctgggtgagcaaaaacaggaaggcaaaatgccgcaaaaaagggaataagggcgacacggaaatgttgaatactcatactcttcctttttcaatattattgaagcatttatcagggttattgtctcatgagcggatacatatttgaatgtatttagaaaaataaacaaataggggttccgcgcacatttccccgaaaagtgccacctgacgt

SEQ ID NO: 8 - DNA, 10704 bp, synthetic construct
  source 1..10704: mol_type = other DNA
gacggatcgggagatctcccgatcccctatggtcgactctcagtacaatctgctctgatgccgcatagttaagccagtatctgctccctgcttgtgtgttggaggtcgctgagtagtgcgcgagcaaaatttaagctacaacaaggcaaggcttgaccgacaattgcatgaagaatctgcttagggttaggcgttttgcgctgcttcgcgatgtacgggccagatatacgcgttgacattgattattgactagttattaatagtaatcaattacggggtcattagttcatagcccatatatggagttccgcgttacataacttacggtaaatggcccgcctggctgaccgcccaacgacccccgcccattgacgtcaataatgacgtatgttcccatagtaacgccaatagggactttccattgacgtcaatgggtggactatttacggtaaactgcccacttggcagtacatcaagtgtatcatatgccaagtacgccccctattgacgtcaatgacggtaaatggcccgcctggcattatgcccagtacatgaccttatgggactttcctacttggcagtacatctacgtattagtcatcgctattaccatggtgatgcggttttggcagtacatcaatgggcgtggatagcggtttgactcacggggatttccaagtctccaccccattgacgtcaatgggagtttgttttggcaccaaaatcaacgggactttccaaaatgtcgtaacaactccgccccattgacgcaaatgggcggtaggcgtgtacggtgggaggtctatataagcagagctggtttagtgaaccgtcagatccgctagcgctaccggtcgccaccatggcctctaattttactcaatttgtgcttgtcgataatggggggacgggagatgtgaccgttgcccctagcaatttcgcaaatggcgttgcagaatggatctctagcaacagcagaagccaagcgtacaaagtaacgtgttccgttcgccaaagctccgcccaaaaacggaagtatacaataaaggttgaggtgccgaaagtagccactcaaacagttggtggggtagaattgcccgtagcggcatggcggtcatatctcaatatggaactcactatcccaatcttcgccacgaatagcgattgtgagctgatagttaaggctatgcaaggtcttctcaaagatggaaaccctattccatctgctatcgccgccaacagcgggatatacagccagaactatccgattgtgcagtccggactcagatctcgagctcaagcttcgaattctgcagtcgacggtaccgcgggcccgggatccatggactcgggccgggacttcctgaccctgcacggcctacaggatgatgaggatctacaggcgctgctgaagggcagccagctcctgaaggtgaagtccagctcatggaggagagagcgcttctacaagttgcaggaggactgcaagaccatctggcaggagtcccgcaaggtcatgcggaccccggagtcccagctgttctccatcgaggacattcaggaggtgcgaatggggcaccgcacggagggtctggagaagttcgcccgtgatgtgcccgaggaccgctgcttctccattgtcttcaaggaccagcgcaatacactagacctcatcgccccatcgccagctgatgcccagcactgggtgctggggctgcacaagatcatccaccactcaggctccatggaccagcgtcagaagctacagcactggattcactcctgcttgcgaaaagctgacaaaaacaaggacaacaagatgagcttcaaggagctgcagaacttcctgaaggagctcaacatccagcctcgagccgaattcaccctggccgccagggccagcgtgctgagcggcggcgagctggacaggtgggagaagatcaggctgaggcccggcggcaagaagaagtataagctgaagcacatcgtgtgggccagcagggagctggagaggttcgccgtgaaccccggcctgctggagaccagcgagggctgcaggcagatcctgggccagctgcagcccagcctgcagaccggcagcgaggagctgaggagcctgtacaacaccgtggccaccctgtactgcgtgcaccagaggatcgagatcaaggacaccaaggaggccctggacaagatcgaggaggagcagaacaagtccaagaagaaggcccagcaggccgccgccgacaccggccacagcagccaggtgagccagaactaccccatcgtgcagaacatccagggccagatggtgcaccaggccatcagccccaggaccctgaacgcctgggtgaaggtggtggaggagaaggccttcagccccgaggtgatccccatgttcagcgccctgagcgagggagccaccccccaggacctgaacaccatgctgaacaccgtgggcggccaccaggccgccatgcagatgctgaaggagaccatcaacgaggaggccgccgagtgggacagggtgcaccccgtgcacgccggccccatcgcccccggccagatgagggagccccgcggcagcgacatcgccggcaccaccagcaccctgcaggagcagatcggctggatgaccaacaacccccccatccccgtgggcgaaatctacaagaggtggatcatcctgggcctgaacaagatcgtgaggatgtacagccccaccagcatcctggatatcaggcagggccccaaagagcccttcagggactacgtggacaggttctacaagaccctgcgcgccgagcaggccagccaggaggtgaagaactggatgaccgagaccctgctggtgcagaacgccaaccccgactgcaagaccatcctgaaggccctgggacccgccgccaccctggaggagatgatgaccgcctgccagggcgtgggcggccccggccacaaggccagggtgctggccgaggccatgagccaggtgaccaacaccgccaccatcatgatgcagaggggcaacttcaggaaccagaggaagatggtgaagtgcttcaactgcggcaaggagggccacaccgccaggaactgccgcgcccccaggaagaagggctgctggaagtgcggcaaggagggccaccagatgaaggactgcaccgagaggcaggctaattttttagggaagatctggccttcctacaagggaaggccagggaattttcttcagagcagaccagagccaacagccccaccatttcttcagagcagaccagagccaacagccccaccagaagagagcttcaggtctggggtagagacaacaactccccctcagaagcaggagccgatagacaaggaactgtatcctttaacttccctcagatcactctttggcaacgacccctcgtcacaataaagatcggtggccagctgaaggaggccctgctggacaccggcgccgacgacaccgtgctggaggagatgagcctgcccggcaggtggaagcccaagatgatcggcggcatcggcggcttcatcaaggtgaggcagtacgaccagatcctgatcgagatctgcggccacaaggccatcggcaccgtgctggtgggacctacacctgtgaacatcatcggcaggaacctgctgacccagatcggctgcaccctgaacttccccatcagccccatcgagaccgtgcccgtgaagctgaagcccggcatggacggccctaaggtgaagcagtggcccctgaccgaggagaagatcaaggccctggtggagatctgcaccgagatggagaaggagggcaagatcagcaagatcggccccgagaacccctacaacacccccgtgttcgccatcaagaagaaggacagcaccaagtggaggaagctggtggacttcagggagctgaacaagaggacccaggacttctgggaggtgcagctgggcatcccccaccccgccggcctgaagaagaagaagagcgtgaccgtgctggacgtgggcgacgcctacttcagcgtgcccctggacgaggacttcaggaagtataccgccttcaccatccccagcatcaacaacgagacccccggcatccgctaccagtacaacgtgctgccccagggctggaagggcagccccgccatcttccagagcagcatgacaaagatcctggagcccttcaagaagcagaaccccgacatcgtgatctatcagtacatggacgacctgtacgtgggcagcgacctggagatcggccagcacaggaccaagatcgaggagctgaggcagcacctgctgaggtggggcctgaccacccccgacaagaagcaccagaaggagcccccattcctgtggatgggctacgagctgcaccccgacaagtggaccgtgcagcccatcgtgctgcccgagaaggacagctggaccgtgaacgacattcagaagctggtgggcaagctgaactgggccagccagatctaccccggcatcaaggtgaggcagctgtgcaagctgctgaggggcacaaaggctctgaccgaggtgatccccctgaccgaggaggccgagctggagctggccgagaacagggagatcctgaaggagcccgtgcacggcgtgtactacgaccccagcaaggacctgatcgccgagatccagaagcagggccagggccagtggacctaccagatctaccaggagcccttcaagaacctgaagaccggcaagtacgcccgcatgcgcggcgcccacaccaacgacgtgaagcagctgaccgaggccgtgcagaagatcaccaccgagagcatcgtgatctggggcaagactcctaagttcaagctgcccatccagaaggagacctgggagacctggtggaccgagtactggcaggccacctggattcccgagtgggagttcgtgaacacccctcccctggtgaagctgtggtatcagctggagaaggagcccatcgtgggcgccgagaccttctacgtggacggcgccgccaacagggagaccaagctgggcaaggccggctacgtgaccaacaagggccgccagaaggtggtgcccctgaccaacaccaccaaccagaagaccgagctgcaggctatctacctggccctgcaggactcaggcctggaggtgaacatcgtgaccgacagccagtacgccctgggcatcatccaggcccagcccgacaagagcgagagcgagctggtgaaccagatcatcgagcagctgatcaagaaggagaaggtgtacctggcctgggtgcccgcccacaagggcatcggcggcaacgagcaggtggacaagctggtgagcgccggcatcaggaagatcctgttcctggacggcatcgacaaggcccaggacgagcacgagaagtaccacagcaactggagggctatggctagcgacttcaacctgcctcccgtggtggctaaggagatcgtggccagctgcgacaagtgccagctgaagggcgaggccatgcacggccaggtggactgcagccccggcatctggcagctggtttgcacccacctggagggcaaggtgatcctggtggccgtgcacgtggcctccggctacatcgaggccgaggtgatccccgccgagaccggccaggagaccgcctacttcctgctgaagctggccggccgctggcccgtgaagaccatccacaccgacaacggcagcaacttcaccagcgccaccgtgaaggccgcctgctggtgggccggcatcaagcaggagttcggcatcccctacaacccccagtctcagggcgtggtggagagcatgaacaaggagctgaagaagatcatcggccaggtgagggaccaggccgagcacctgaagaccgccgtgcagatggccgtgttcatccacaacttcaagaggaagggcggcatcggcggctacagcgccggcgagaggatcgtggacatcatcgccaccgacatccagaccaaggagctgcagaagcagatcaccaagatccagaacttcagggtgtactacagggacagcaggaaccctctgtggaagggccccgccaagctgctgtggaagggcgagggcgccgtggtgatccaggacaacagcgacatcaaggtggtgcccaggaggaaggccaagatcatcagggactacggcaagcagatggccggcgacgactgcgtggcctccaggcaggacgaggactgactcgagcatgcatctagagggccctattctatagtgtcacctaaatgctagagctcgctgatcagcctcgactgtgccttctagttgccagccatctgttgtttgcccctcccccgtgccttccttgaccctggaaggtgccactcccactgtcctttcctaataaaatgaggaaattgcatcgcattgtctgagtaggtgtcattctattctggggggtggggtggggcaggacagcaagggggaggattgggaagacaatagcaggcatgctggggatgcggtgggctctatggcttctgaggcggaaagaaccagctggggctctagggggtatccccacgcgccctgtagcggcgcattaagcgcggcgggtgtggtggttacgcgcagcgtgaccgctacacttgccagcgccctagcgcgcgctcctttcgctttcttcccttcctttctcgccacgttcgccggctttccccgtcaagctctaaatcggggcatccctttagggttccgatttagtgctttacggcacctcgaccccaaaaaacttgattagggtgatggttcacgtagtgggccatcgccctgatagacggtttttcgccctttgacgttggagtccacgttctttaatagtggactcttgttccaaactggaacaacactcaaccctatctcggtctattcttttgatttataagggattttggggatttcggcctattggttaaaaaatgagctgatttaacaaaaatttaacgcgaattaattctgtggaatgtgtgtcagttagggtgtggaaagtccccaggctccccaggcaggcagaagtatgcaaagcatgcatctcaattagtcagcaaccaggtgtggaaagtccccaggctccccagcaggcagaagtatgcaaagcatgcatctcaattagtcagcaaccatagtcccgcccctaactccgcccatcccgcccctaactccgcccagttccgcccattctccgccccatggctgactaattttttttatttatgcagaggccgaggccgcctctgcctctgagctattccagaagtagtgaggaggcttttttggaggcctaggcttttgcaaaaagctcccgggagcttgtatatccattttcggatctgatcaagagacaggatgaggatcgtttcgcatgattgaacaagatggattgcacgcaggttctccggccgcttgggtggagaggctattcggctatgactgggcacaacagacaatcggctgctctgatgccgccgtgttccggctgtcagcgcaggggcgcccggttctttttgtcaagaccgacctgtccggtgccctgaatgaactgcaggacgaggcagcgcggctatcgtggctggccacgacgggcgttccttgcgcagctgtgctcgacgttgtcactgaagcgggaagggactggctgctattgggcgaagtgccggggcaggatctcctgtcatctcaccttgctcctgccgagaaagtatccatcatggctgatgcaatgcggcggctgcatacgcttgatccggctacctgcccattcgaccaccaagcgaaacatcgcatcgagcgagcacgtactcggatggaagccggtcttgtcgatcaggatgatctggacgaagagcatcaggggctcgcgccagccgaactgttcgccaggctcaaggcgcgcatgcccgacggcgaggatctcgtcgtgacccatggcgatgcctgcttgccgaatatcatggtggaaaatggccgcttttctggattcatcgactgtggccggctgggtgtggcggaccgctatcaggacatagcgttggctacccgtgatattgctgaagagcttggcggcgaatgggctgaccgcttcctcgtgctttacggtatcgccgctcccgattcgcagcgcatcgccttctatcgccttcttgacgagttcttctgagcgggactctggggttcgaaatgaccgaccaagcgacgcccaacctgccatcacgagatttcgattccaccgccgccttctatgaaaggttgggcttcggaatcgttttccgggacgccggctggatgatcctccagcgcggggatctcatgctggagttcttcgcccaccccaacttgtttattgcagcttataatggttacaaataaagcaatagcatcacaaatttcacaaataaagcatttttttcactgcattctagttgtggtttgtccaaactcatcaatgtatcttatcatgtctgtataccgtcgacctctagctagagcttggcgtaatcatggtcatagctgtttcctgtgtgaaattgttatccgctcacaattccacacaacatacgagccggaagcataaagtgtaaagcctggggtgcctaatgagtgagctaactcacattaattgcgttgcgctcactgcccgctttccagtcgggaaacctgtcgtgccagctgcattaatgaatcggccaacgcgcggggagaggcggtttgcgtattgggcgctcttccgcttcctcgctcactgactcgctgcgctcggtcgttcggctgcggcgagcggtatcagctcactcaaaggcggtaatacggttatccacagaatcaggggataacgcaggaaagaacatgtgagcaaaaggccagcaaaaggccaggaaccgtaaaaaggccgcgttgctggcgtttttccataggctccgcccccctgacgagcatcacaaaaatcgacgctcaagtcagaggtggcgaaacccgacaggactataaagataccaggcgtttccccctggaagctccctcgtgcgctctcctgttccgaccctgccgcttaccggatacctgtccgcctttctcccttcgggaagcgtggcgctttctcaatgctcacgctgtaggtatctcagttcggtgtaggtcgttcgctccaagctgggctgtgtgcacgaaccccccgttcagcccgaccgctgcgccttatccggtaactatcgtcttgagtccaacccggtaagacacgacttatcgccactggcagcagccactggtaacaggattagcagagcgaggtatgtaggcggtgctacagagttcttgaagtggtggcctaactacggctacactagaaggacagtatttggtatctgcgctctgctgaagccagttaccttcggaaaaagagttggtagctcttgatccggcaaacaaaccaccgctggtagcggtggtttttttgtttgcaagcagcagattacgcgcagaaaaaaaggatctcaagaagatcctttgatcttttctacggggtctgacgctcagtggaacgaaaactcacgttaagggattttggtcatgagattatcaaaaaggatcttcacctagatccttttaaattaaaaatgaagttttaaatcaatctaaagtatatatgagtaaacttggtctgacagttaccaatgcttaatcagtgaggcacctatctcagcgatctgtctatttcgttcatccatagttgcctgactccccgtcgtgtagataactacgatacgggagggcttaccatctggccccagtgctgcaatgataccgcgagacccacgctcaccggctccagatttatcagcaataaaccagccagccggaagggccgagcgcagaagtggtcctgcaactttatccgcctccatccagtctattaattgttgccgggaagctagagtaagtagttcgccagttaatagtttgcgcaacgttgttgccattgctacaggcatcgtggtgtcacgctcgtcgtttggtatggcttcattcagctccggttcccaacgatcaaggcgagttacatgatcccccatgttgtgcaaaaaagcggttagctccttcggtcctccgatcgttgtcagaagtaagttggccgcagtgttatcactcatggttatggcagcactgcataattctcttactgtcatgccatccgtaagatgcttttctgtgactggtgagtactcaaccaagtcattctgagaatagtgtatgcggcgaccgagttgctcttgcccggcgtcaatacgggataataccgcgccacatagcagaactttaaaagtgctcatcattggaaaacgttcttcggggcgaaaactctcaaggatcttaccgctgttgagatccagttcgatgtaacccactcgtgcacccaactgatcttcagcatcttttactttcaccagcgtttctgggtgagcaaaaacaggaaggcaaaatgccgcaaaaaagggaataagggcgacacggaaatgttgaatactcatactcttcctttttcaatattattgaagcatttatcagggttattgtctcatgagcggatacatatttgaatgtatttagaaaaataaacaaataggggttccgcgcacatttccccgaaaagtgccacctgacgtc

SEQ ID NO: 9 - protein, 982 aa, Sindbis virus
MSAAPLVTAMCLLGNVSFPCDRPPTCYTREPSRALDILEENVNHEAYDTLLNAILRCGSSGRSKRSVIDDFTLTSPYLGTCSYCHHTVPCFSPVKIEQVWDEADDNTIRIQTSAQFGYDQSGAASANKYRYMSLKQDHTVKEGTMDDIKISTSGPCRRLSYKGYFLLAKCPPGDSVTVSIVSSNSATSCTLARKIKPKFVGREKYDLPPVHGKKIPCTVYDRLKETTAGYITMHRPRPHAYTSYLEESSGKVYAKPPSGKNITYECKCGDYKTGTVSTRTEITGCTAIKQCVAYKSDQTKWVFNSPDLIRHDDHTAQGKLHLPFKLIPSTCMVPVAHAPNVIHGFKHISLQLDTDHLTLLTTRRLGANPEPTTEWIVGKTVRNFTVDRDGLEYIWGNHEPVRVYAQESAPGDPHGWPHEIVQHYYHRHPVYTILAVASATVAMMIGVTVAVLCACKARRECLTPYALAPNAVIPTSLALLCCVRSANAETFTETMSYLWSNSQPFFWVQLCIPLAAFIVLMRCCSCCLPFLVVAGAYLAKVDAYEHATTVPNVPQIPYKALVERAGYAPLNLEITVMSSEVLPSTNQEYITCKFTTVVPSPKIKCCGSLECQPAAHADYTCKVFGGVYPFMWGGAQCFCDSENSQMSEAYVELSADCASDHAQAIKVHTAAMKVGLRIVYGNTTSFLDVYVNGVTPGTSKDLKVIAGPISASFTPFDHKVVIHRGLVYNYDFPEYGAMKPGAFGDIQATSLTSKDLIASTDIRLLKPSAKNVHVPYTQASSGFEMWKNNSGRPLQETAPFGCKIAVNPLRAVDCSYGNIPISIDIPNAAFIRTSDAPLVSTVKCEVSECTYSADFGGMATLQYVSDREGQCPVHSHSSTATLQESTVHVLEKGAVTVHFSTASPQANFIVSLCGKKTTCNAECKPPADHIVSTPHKNDQEFQAAISKTSWSWLFALFGGASSLLIIGLMIFACSMMLTSTRR

SEQ ID NO: 10 - DNA, 5822 bp, synthetic construct
  source 1..5822: mol_type = other DNA
tttaaatacatcattgcaatgaaaataaatgttttttattaggcagaatccagatgctcaaggcccttcataatatcccccagtttagtagttggacttagggaacaaaggaacctttaatagaaattggacagcaagaaagcgagcttagtgatacttgtgggccagggcattagccacaccagccaccactttctgataggcagcctgcactggtggggtgaattccgtttttttttttttttttcataaaaattaaaaactcaaatataattgaggcctctttgagcatggtatcacaagttgatttggtccaaacatgaagaatctgttgtgcaggatttgagttactttccaagtcggttcatctctatgtctgtataaatctgtcttttcttggtgtgctttaatttaatgcaaagatggataccaactcggagaaccaagaatagtccaatgattaaccctatgataaagaaaaaagaggcaatagagcttttccaactactgaaccaaccttctacaagctcgattggatttttggatagcccagtatcaccaaaaaataaactctcatcatcaggaagttgcgaagcagcgtcttgaatgtgaggatgttcgaacacctgagcctttgagctaagatgaagatcggagtccaacataccatgtccaatcatgtataaaggaaacttatatcctgaactggtcctcagaactccattgggtccaatttccacgtcttcatatggtgcccagtcatcccacagttccctttctgtggtagttccactgatcattccgaccattcttgagaggattggagcagcaatatcgactctgatgtatctggtctcaaagtattttagggtaccattgattatggtgaaagcaggaccggttcctgggtttttaggagcaagatagctgagatccactggagagattggaagacccgctctgattttgctccaggtttcttggcagagggaataatccaagatcctctcaacgtcctgaattagacttacatccactgaggtctgagatggagcagagatacttgacccttctgggcattcagggaatctggctgcagcaaagagatccttatcagccatctcgaaccagacacctgatgggagtctgactccccaatgcttgcagtattgcattttgcaggccttgcctccagtttcataagcaaagtagttacttctgaaccctgtgccctcctttcccagggatgatagctctccgtcctctgagaagaaggtgatgtccatggaaatgaggttagaatcacatagccctttgaccttatagtcagaatgccaggttgtagagttatggacagtggggcatatgtaattgctgcattttccgttgatgaactgtgaatcaacccattctcctgtgtattcatcaaccagcacatggtgaggagtcacctggacaatcactgcttcggcatccgtcacagttgcatatccacaactttgaggagggaagcctggattcagccaagttccttgtttcgtttgttcaatgctttccttgcattgttctacagatggagtgaaggatcggatggaatgtgttatatacttcggtccataccagcggaaatcacaagtagtgacccatttggaagcatgacacatccaaccgtctgcttgaatagccttgtgactcttgggcattttgacttgtaaggctgtgcctattaagtcattatgccaatttaaatctgagcttgacgggcaataatggtaattagaaggaacatttttccagtttcctttttggttgtgtggaaaaactatggtgaacttgcaattcaccccaatgaataaaaaggctaagtacaaaaggcacttcatagtgtcagaattcagatctcacgtgctttgccaaagtgatgggccagcacacagaccagcacgttgcccaggagctgtgggaggaagataagaggtatgaacatgattagcaaaagggcctagcttggactcagaataatccagccttatcccaaccataaaataaaagcagaatggtagctggattgtagctgctattagcaatatgaaacctcttacatcagttacaatttatatgcagaaatatttatatgcagaaatattgctattgccttaacccagaaattatcactgttattctttagaatggtgcaaagaggcatgatacattgtatcattattgccctgaaagaaagagattagggaaagtattagaaataagataaacaaaaaagtatattaaaagaagaaagcattttttaaaattacaaatgcaaaattaccctgatttggtcaatatgtgtaccctgttacttctccccttcctatgacatgaacttaaccatagaaaagaaggggaaagaaaacatcaagggtcccatagactcaccctgaagttctcaggatccgagctcggtaccacatgtaagcttcgaggggaggctggatcggtcccggtgtcttctatggaggtcaaaacagcgtggatggcgtctccaggcgatctgacggttcactaaacgagctctgcttatatagacctcccaccgtacacgcctaccgcccatttgcgtcaatggggcggagttgttacgacattttggaaagtcccgttgattttggtgccaaaacaaactcccattgacgtcaatggggtggagacttggaaatccccgtgagtcaaaccgctatccacgcccattgatgtactgccaaaaccgcatcaccatggtaatagcgatgactaatacgtagatgtactgccaagtaggaaagtcccataaggtcatgtactgggcataatgccaggcgggccatttaccgtcattgacgtcaatagggggcgtacttggcatatgatacacttgatgtactgccaagtgggcagtttaccgtaaatactccacccattgacgtcaatggaaagtccctattggcgttactatgggaacatacgtcattattgacgtcaatgggcgggggtcgttgggcggtcagccaggcgggccatttaccgtaagttatgtaacgcggaactccatatatgggctatgaactaatgaccccgtaattgattactattaataactagtcaataatcaatgtcaacatggcggtaatgttggacatgagccaatataaatgtacatattatgatatggatacaacgtatgcaatgggccaagctcatggctgactaattttttttatttatgcagaggccgaggccggatcctctagcccatgggggccccctcaggggatccacgtcaggtggcacttttcggggaaatgtgcgcggaacccctatttgtttatttttctaaatacattcaaatatgtatccgctcatgagacaataaccctgataaatgcttcaataatattgaaaaaggaagagtatgagtattcaacatttccgtgtcgcccttattcccttttttgcggcattttgccttcctgtttttgctcacccagaaacgctggtgaaagtaaaagatgctgaagatcagttgggtgcacgagtgggttacatcgaactggatctcaacagcggtaagatccttgagagttttcgccccgaagaacgttttccaatgatgagcacttttaaagttctgctatgtggcgcggtattatcccgtattgacgccgggcaagagcaactcggtcgccgcatacactattctcagaatgacttggttgagtactcaccagtcacagaaaagcatcttacggatggcatgacagtaagagaattatgcagtgctgccataaccatgagtgataacactgcggccaacttacttctgacaacgatcggaggaccgaaggagctaaccgcttttttgcacaacatgggggatcatgtaactcgccttgatcgttgggaaccggagctgaatgaagccataccaaacgacgagcgtgacaccacgatgcctgtagcaatggcaacaacgttgcgcaaactattaactggcgaactacttactctagcttcccggcaacaattaatagactggatggaggcggataaagttgcaggaccacttctgcgctcggcccttccggctggctggtttattgctgataaatctggagccggtgagcgtgggtctcgcggtatcattgcagcactggggccagatggtaagccctcccgtatcgtagttatctacacgacggggagtcaggcaactatggatgaacgaaatagacagatcgctgagataggtgcctcactgattaagcattggtaactgtcagaccaagtttactcatatatactttagattgatttaaaacttcatttttaatttaaaaggatctaggtgaagatcctttttgataatctcatgaccaaaatcccttaacgtgagttttcgttccactgagcgtcagaccccgtagaaaagatcaaaggatcttcttgagatcctttttttctgcgcgtaatctgctgcttgcaaacaaaaaaaccaccgctaccagcggtggtttgtttgccggatcaagagctaccaactctttttccgaaggtaactggcttcagcagagcgcagataccaaatactgttcttctagtgtagccgtagttaggccaccacttcaagaactctgtagcaccgcctacatacctcgctctgctaatcctgttaccagtggctgctgccagtggcgataagtcgtgtcttaccgggttggactcaagacgatagttaccggataaggcgcagcggtcgggctgaacggggggttcgtgcacacagcccagcttggagcgaacgacctacaccgaactgagatacctacagcgtgagctatgagaaagcgccacgcttcccgaagggagaaaggcggacaggtatccggtaagcggcagggtcggaacaggagagcgcacgagggagcttccagggggaaacgcctggtatctttatagtcctgtcgggtttcgccacctctgacttgagcgtcgatttttgtgatgctcgtcaggggggcggagcctatggaaaaacgccagcaacgcggcctttttacggttcctggccttttgctggccttttgctcacatgttctttcctgcgttatcccctgattctgtggataaccgtattaccgcctttgagtgagctgataccgctcgccgcagccgaacgaccgagcgcagcgagtcagtgagcgaggaagcagatctgcggccgcactagtgctagactgccatgtcgagggattccgggtcactgtgagtgggggaggcagggaagaagggctcacaggacagtcaaaccatgccccctgtttttccttcttcaagtagacctctataagacaacagagacaactaaggctgagtggccaggcgaggagaaaccatctcgccgtaaaacatggaaggaacacttcaggggaaaggtggtatctctaagcaagagaactgagtggagtcaaggctgagagatgcaggataagcaaatgggtagtgaaaagacattcatgaggacagctaaaacaataagtaatgtaaaatacagcatagcaaaactttaacctccaaatcaagcctctacttgaatccttttctgagggatgaataaggcataggcatcaggggctgttgccaatgtgcattagctgtttgcagcctcaccttctttcatggagtttaagatatagtgtattttcccaaggtttgaactagctcttcatttctttatgttttaaatgcactgacctcccacattccctttttagtaaaatattcagaaataa

SEQ ID NO: 11 - DNA, 21 bp, synthetic construct
  source 1..21: mol_type = other DNA
acagatgagatgatcgcccag

SEQ ID NO: 12 - DNA, 20 bp, synthetic construct
  source 1..20: mol_type = other DNA
tctgcatggcgaaagggatc

SEQ ID NO: 13 - DNA, 21 bp, synthetic construct
  source 1..21: mol_type = other DNA
aggtcggtgtgaacggatttg

SEQ ID NO: 14 - DNA, 23 bp, synthetic construct
  source 1..23: mol_type = other DNA
tgtagaccatgtagttgaggtca

SEQ ID NO: 15 - DNA, 7961 bp, synthetic construct
  source 1..7961: mol_type = other DNA
tcgcgcgtttcggtgatgacggtgaaaacctctgacacatgcagctcccggagacggtcacagcttgtctgtaagcggatgccgggagcagacaagcccgtcagggcgcgtcagcgggtgttggcgggtgtcggggctggcttaactatgcggcatcagagcagattgtactgagagtgcaccatatgcggtgtgaaataccgcacagatgcgtaaggagaaaataccgcatcaggcgccattcgccattcaggctgcgcaactgttgggaagggcgatcggtgcgggcctcttcgctattacgccagctggcgaaagggggatgtgctgcaaggcgattaagttgggtaacgccagggttttcccagtcacgacgttgtaaaacgacggccagtgaattcgagcttgcatgcctgcaggtcgttacataacttacggtaaatggcccgcctggctgaccgcccaacgacccccgcccattgacgtcaataatgacgtatgttcccatagtaacgccaatagggactttccattgacgtcaatgggtggactatttacggtaaactgcccacttggcagtacatcaagtgtatcatatgccaagtacgccccctattgacgtcaatgacggtaaatggcccgcctggcattatgcccagtacatgaccttatgggactttcctacttggcagtacatctacgtattagtcatcgctattaccatggtgatgcggttttggcagtacatcaatgggcgtggatagcggtttgactcacggggatttccaagtctccaccccattgacgtcaatgggagtttgttttggcaccaaaatcaacgggactttccaaaatgtcgtaacaactccgccccattgacgcaaatgggcggtaggcgtgtacggtgggaggtctatataagcagagctcgtttagtgaaccgtcagatcgcctggagacgccatccacgctgttttgacctccatagaagacaccgggaccgatccagcctccggactctagaggatccggtactcgaggaactgaaaaaccagaaagttaactggtaagtttagtctttttgtcttttatttcaggtcccgatccggtggtggtgcaaatcaaagaactgctcctcagtggatgttgcctttacttctaggcctgtacggaagtgttacttctgctctaaaagctgcggaattgtacccgcggagccaccatgcaccagggcgccccctcgtgggggcgccggtggttcgtcgtatgggcgctcttggggttgacgctgggggtcctggtggcgtcggcggctccgagttcccccggcacgcctggggtcgcggccgcgacccaggcggcgaacgggggccctgccactccggcgccgcccgcccttggcgccgccccaacgggggacccgaaaccgaagaagaacaaaaaaccgaaaaacccaacgccaccacgccccgccggcgacaacgcgaccgtcgccgcgggccacgccaccctgcgcgagcacctgcgggacatcaaggcggagaacaccgatgcaaacttttacgtgtgcccaccccccacgggcgccacggtggtgcagttcgagcagccgcgccgctgcccgacccggcccgagggtcagaactacacggagggcatcgcggtggtcttcaaggagaacatcgccccgtacaagttcaaggccaccatgtactacaaagacgtcaccgtttcgcaggtgtggttcggccaccgctactcccagtttatggggatctttgaggaccgcgcccccgtccccttcgaggaggtgatcgacaagatcaacgccaagggggtctgtcggtccacggccaagtacgtgcgcaacaacctggagaccaccgcgtttcaccgggacgaccacgagaccgacatggagctgaaaccggccaacgccgcgacccgcacgagccggggctggcacaccaccgacctcaagtacaacccctcgcgggtggaggcgttccaccggtacgggacgacggtaaactgcatcgtcgaggaggtggacgcgcgctcggtgtacccgtacgacgagtttgtgctggcgactggcgactttgtgtacatgtccccgttttacggctaccgggaggggtcgcacaccgaacacaccagctacgccgccgaccgcttcaagcaggtcgacggcttctacgcgcgcgacctcaccaccaaggcccgggccacggcgccgaccacccggaacctgctcacgacccccaagttcaccgtggcctgggactgggtgccaaagcgcccgtcggtctgcaccatgaccaagtggcaggaagtggacgagatgctgcgctccgagtacggcggctccttccgattctcctccgacgccatatccaccaccttcaccaccaacctgaccgagtacccgctctcgcgcgtggacctgggggactgcatcggcaaggacgcccgcgacgccatggaccgcatcttcgcccgcaggtacaacgcgacgcacatcaaggtgggccagccgcagtactacctggccaatgggggctttctgatcgcgtaccagccccttctcagcaacacgctcgcggagctgtacgtgcgggaacacctccgagagcagagccgcaagcccccaaaccccacgcccccgccgcccggggccagcgccaacgcgtccgtggagcgcatcaagaccacctcctccatcgagttcgcccggctgcagtttacgtacaaccacatacagcgccatgtcaacgatatgttgggccgcgttgccatcgcgtggtgcgagctacagaatcacgagctgaccctgtggaacgaggcccgcaagctgaaccccaacgccatcgcctcggtcaccgtgggccggcgggtgagcgcgcggatgctcggcgacgtgatggccgtctccacgtgcgtgccggtcgccgcggacaacgtgatcgtccaaaactcgatgcgcatcagctcgcggcccggggcctgctacagccgccccctggtcagctttcggtacgaagaccagggcccgttggtcgaggggcagctgggggagaacaacgagctgcggctgacgcgcgatgcgatcgagccgtgcaccgtgggacaccggcgctacttcaccttcggtgggggctacgtgtacttcgaggagtacgcgtactcccaccagctgagccgcgccgacatcaccaccgtcagcaccttcatcgacctcaacatcaccatgctggaggatcacgagtttgtccccctggaggtgtacacccgccacgagatcaaggacagcggcctgctggactacacggaggtccagcgccgcaaccagctgcacgacctgcgcttcgccgacatcgacacggtcatccacgccgacgccaacgccgccatgttcgcgggcctgggcgcgttcttcgaggggatgggcgacctggggcgcgcggtcggcaaggtggtgatgggcatcgtgggcggcgtggtatcggccgtgtcgggcgtgtcctccttcatgtccaacccctttggggcgctggccgtgggtctgttggtcctggccggcctggcggcggccttcttcgcctttcgttacgtcatgcggctgcagagcaaccccatgaaggccctgtaccctctaaccaccaaggagctcaagaaccccaccaacccggacgcgtccggggagggcgaggagggcggcgactttgacgaggccaagctagccgaggccagggagatgatacggtacatggccctggtgtcggccatggagcgcacggaacacaaggccaagaagaagggcacgagcgcgctgctcagcgccaaggtcaccgacatggtcatgcgcaagcgccgcaacaccaactacacccaagttcccaacaaagacggtgacgccgacgaggacgacctggcaacaaacttctctctgctgaaacaagccggagatgtcgaagagaatcctggaccgatggggggggctgccgccaggttgggggccgtgattttgtttgtcgtcatagtgggcctccatggggtccgcggcaaatatgccttggcggatgcctctctcaagatggccgaccccaatcgctttcgcggcaaagaccttccggtcctggaccagctgaccgaccctccgggggtccggcgcgtgtaccacatccaggcgggcctaccggacccgttccagccccccagcctcccgatcacggtttactacgccgtgttggagcgcgcctgccgcagcgtgctcctaaacgcaccgtcggaggccccccagattgtccgcggggcctccgaagacgtccggaaacaaccctacaacctgaccatcgcttggtttcggatgggaggcaactgtgctatccccatcacggtcatggagtacaccgaatgctcctacaacaagtctctgggggcctgtcccatccgaacgcagccccgctggaactactatgacagcttcagcgccgtcagcgaggataacctggggttcctgatgcacgcccccgcgtttgagaccgccggcacgtacctgcggctcgtgaagataaacgactggacggagattacacagtttatcctggagcaccgagccaagggctcctgtaagtacgccctcccgctgcgcatccccccgtcagcctgcctctccccccaggcctaccagcagggggtgacggtggacagcatcgggatgctgccccgcttcatccccgagaaccagcgcaccgtcgccgtatacagcttgaagatcgccgggtggcacgggcccaaggccccatacacgagcaccctgctgcccccggagctgtccgagacccccaacgccacgcagccagaactcgccccggaagaccccgaggattcggccctcttggaggaccccgtggggacggtggcgccgcaaatcccaccaaactggcacatcccgtcgatccaggacgccgcgacgccttaccatcccccggccaccccgaacaacatgggcctgatcgccggcgcggtgggcggcagtctcctggcagccctggtcatttgcggaattgtgtactggatgcaccgccgcactcggaaagccccaaagcgcatacgcctcccccacatccgggaagacgaccagccgtcctcgcaccagcccttgttttactagccggtcttgcagcacatacatgaggatcacccatgtctgcaggtcgactctagaaaacatgaggatcacccatgtctgcagtattcccgggttcattagatcctaaggtacctaattgcctagaaaacatgaggatcacccatgtctgcaggtcgactctagaaaacatgaggatcacccatgtctgcagtattcccgggttcattagatcctaaggtacctaattgcctagaaaacatgaggatcacccatgtctgcaggtcgactctagaaaacatgaggatcacccatgtgtgcaccttaagcttggcccgcggggatccagacatgataagatacattgatgagtttggacaaaccacaactagaatgcagtgaaaaaaatgctttatttgtgaaatttgtgatgctattgctttatttgtaaccattataagctgcaataaacaagttaacaacaacaattgcattcattttatgtttcaggttcagggggaggtgtgggaggttttttcggatcctctagagtcgacctgcaggcatgcaagcttggcgtaatcatggtcatagctgtttcctgtgtgaaattgttatccgctcacaattccacacaacatacgagccggaagcataaagtgtaaagcctggggtgcctaatgagtgagctaactcacattaattgcgttgcgctcactgcccgctttccagtcgggaaacctgtcgtgccagctgcattaatgaatcggccaacgcgcggggagaggcggtttgcgtattgggcgctcttccgcttcctcgctcactgactcgctgcgctcggtcgttcggctgcggcgagcggtatcagctcactcaaaggcggtaatacggttatccacagaatcaggggataacgcaggaaagaacatgtgagcaaaaggccagcaaaaggccaggaaccgtaaaaaggccgcgttgctggcgtttttccataggctccgcccccctgacgagcatcacaaaaatcgacgctcaagtcagaggtggcgaaacccgacaggactataaagataccaggcgtttccccctggaagctccctcgtgcgctctcctgttccgaccctgccgcttaccggatacctgtccgcctttctcccttcgggaagcgtggcgctttctcatagctcacgctgtaggtatctcagttcggtgtaggtcgttcgctccaagctgggctgtgtgcacgaaccccccgttcagcccgaccgctgcgccttatccggtaactatcgtcttgagtccaacccggtaagacacgacttatcgccactggcagcagccactggtaacaggattagcagagcgaggtatgtaggcggtgctacagagttcttgaagtggtggcctaactacggctacactagaaggacagtatttggtatctgcgctctgctgaagccagttaccttcggaaaaagagttggtagctcttgatccggcaaacaaaccaccgctggtagcggtggtttttttgtttgcaagcagcagattacgcgcagaaaaaaaggatctcaagaagatcctttgatcttttctacggggtctgacgctcagtggaacgaaaactcacgttaagggattttggtcatgagattatcaaaaaggatcttcacctagatccttttaaattaaaaatgaagttttaaatcaatctaaagtatatatgagtaaacttggtctgacagttaccaatgcttaatcagtgaggcacctatctcagcgatctgtctatttcgttcatccatagttgcctgactccccgtcgtgtagataactacgatacgggagggcttaccatctggccccagtgctgcaatgataccgcgagacccacgctcaccggctccagatttatcagcaataaaccagccagccggaagggccgagcgcagaagtggtcctgcaactttatccgcctccatccagtctattaattgttgccgggaagctagagtaagtagttcgccagttaatagtttgcgcaacgttgttgccattgctacaggcatcgtggtgtcacgctcgtcgtttggtatggcttcattcagctccggttcccaacgatcaaggcgagttacatgatcccccatgttgtgcaaaaaagcggttagctccttcggtcctccgatcgttgtcagaagtaagttggccgcagtgttatcactcatggttatggcagcactgcataattctcttactgtcatgccatccgtaagatgcttttctgtgactggtgagtactcaaccaagtcattctgagaatagtgtatgcggcgaccgagttgctcttgcccggcgtcaatacgggataataccgcgccacatagcagaactttaaaagtgctcatcattggaaaacgttcttcggggcgaaaactctcaaggatcttaccgctgttgagatccagttcgatgtaacccactcgtgcacccaactgatcttcagcatcttttactttcaccagcgtttctgggtgagcaaaaacaggaaggcaaaatgccgcaaaaaagggaataagggcgacacggaaatgttgaatactcatactcttcctttttcaatattattgaagcatttatcagggttattgtctcatgagcggatacatatttgaatgtatttagaaaaataaacaaataggggttccgcgcacatttccccgaaaagtgccacctgacgtctaagaaaccattattatcatgacattaacctataaaaataggcgtatcacgaggccctttcgtc

SEQ ID NO: 16 - DNA, 20 bp, synthetic construct
  source 1..20: mol_type = other DNA
tacaacctgaccatcgcttg

SEQ ID NO: 17 - DNA, 20 bp, synthetic construct
  source 1..20: mol_type = other DNA
gcccccagagacttgttgta

SEQ ID NO: 18 - protein, 982 aa, synthetic construct
MSAAPLVTAMCLLGNVSFPCDRPPTCYTREPSRALDILEENVNHEAYDTLLNAILRCGSSGSVIDDFTLTSPYLGTCSYCHHTVPCFSPVKIEQVWDEADDNTIRIQTSAQFGYDQSGAASANKYRYMMYPYDVPDYATVKEGTMDDIKISTSGPCRRLSYKGYFLLAKCPPGDSVTVSIVSSNSATSCTLARKIKPKFVGREKYDLPPVHGKKIPCTVYDRLAATTAGYITMHRPRPHAYTSYLEESSGKVYAKPPSGKNITYECKCGDYKTGTVSTRTEITGCTAIKQCVAYKSDQTKWVFNSPDLIRHDDHTAQGKLHLPFKLIPSTCMVPVAHAPNVIHGFKHISLQLDTDHLTLLTTRRLGANPEPTTEWIVGKTVRNFTVDRDGLEYIWGNHEPVRVYAQESAPGDPHGWPHEIVQHYYHRHPVYTILAVASATVAMMIGVTVAVLCACKARRECLTPYALAPNAVIPTSLALLCCVRSANAETFTETMSYLWSNSQPFFWVQLCIPLAAFIVLMRCCSCCLPFLVVAGAYLAKVDAYEHATTVPNVPQIPYKALVERAGYAPLNLEITVMSSEVLPSTNQEYITCKFTTVVPSPKIKCCGSLECQPAAHADYTCKVFGGVYPFMWGGAQCFCDSENSQMSEAYVELSADCASDHAQAIKVHTAAMKVGLRIVYGNTTSFLDVYVNGVTPGTSKDLKVIAGPISASFTPFDHKVVIHRGLVYNYDFPEYGAMKPGAFGDIQATSLTSKDLIASTDIRLLKPSAKNVHVPYTQASSGFEMWKNNSGRPLQETAPFGCKIAVNPLRAVDCSYGNIPISIDIPNAAFIRTSDAPLVSTVKCEVSECTYSADFGGMATLQYVSDREGQCPVHSHSSTATLQESTVHVLEKGAVTVHFSTASPQANFIVSLCGKKTTCNAECKPPADHIVSTPHKNDQEFQAAISKTSWSWLFALFGGASSLLIIGLMIFACSMMLTSTRR